European Patent Application EP 4 501 363 A1, published February 5, 2025. Title: 抗B7H4抗体药物偶联物及其用途. Applicant: 映恩生物制药（苏 州）有限公司. The sequence listing filed with the application follows.

SEQUENCE LISTING (10 sequences)

SEQ ID NO: 1 - protein, 5 aa, synthetic construct
SFGMH

SEQ ID NO: 2 - protein, 17 aa, synthetic construct
VISYDASNEYYADSVKG

SEQ ID NO: 3 - protein, 10 aa, synthetic construct
GGALRWYFAY

SEQ ID NO: 4 - protein, 11 aa, synthetic construct
RASQSISSNLG

SEQ ID NO: 5 - protein, 7 aa, synthetic construct
GASTRAT

SEQ ID NO: 6 - protein, 10 aa, synthetic construct
QQYRSWPPLT

SEQ ID NO: 7 - protein, 119 aa, synthetic construct
QVQLVESGGGVVQPGRSLRLSCAASGFTFRSFGMHWVRQAPGKGLEWVAVISYDASNEYYADSVKGRFIISRDNSKDTLYLQMNSLRAGDTAVYYCAKGGALRWYFAYWGQGTLVTVSS

SEQ ID NO: 8 - protein, 108 aa, synthetic construct
EIVMTQSPATLSVSPGERATLSCRASQSISSNLGWYQQKPGQAPRLLIYGASTRATGIPARFSGSGSGTEFTLTISSLQSEDFAVYYCQQYRSWPPLTFGGGTKVEIK

SEQ ID NO: 9 - protein, 449 aa, synthetic construct
QVQLVESGGGVVQPGRSLRLSCAASGFTFRSFGMHWVRQAPGKGLEWVAVISYDASNEYYADSVKGRFIISRDNSKDTLYLQMNSLRAGDTAVYYCAKGGALRWYFAYWGQGTLVTVSSASTKGPSVFPLAPSSKSTSGGTAALGCLVKDYFPEPVTVSWNSGALTSGVHTFPAVLQSSGLYSLSSVVTVPSSSLGTQTYICNVNHKPSNTKVDKKVEPKSCDKTHTCPPCPAPELLGGPSVFLFPPKPKDTLMISRTPEVTCVVVDVSHEDPEVKFNWYVDGVEVHNAKTKPREEQYNSTYRVVSVLTVLHQDWLNGKEYKCKVSNKALPAPIEKTISKAKGQPREPQVYTLPPSREEMTKNQVSLTCLVKGFYPSDIAVEWESNGQPENNYKTTPPVLDSDGSFFLYSKLTVDKSRWQQGNVFSCSVMHEALHNHYTQKSLSLSPGK

SEQ ID NO: 10 - protein, 215 aa, synthetic construct
EIVMTQSPATLSVSPGERATLSCRASQSISSNLGWYQQKPGQAPRLLIYGASTRATGIPARFSGSGSGTEFTLTISSLQSEDFAVYYCQQYRSWPPLTFGGGTKVEIKRTVAAPSVFIFPPSDEQLKSGTASVVCLLNNFYPREAKVQWKVDNALQSGNSQESVTEQDSKDSTYSLSSTLTLSKADYEKHKVYACEVTHQGLSSPVTKSFNRGEC